European Patent Application EP 4 218 930 A1, published August 2, 2023. Title: Treatment and prognosis of cancer. Applicant: Cancerappy, SL. The sequence listing filed with the application follows.

SEQUENCE LISTING (2 sequences)

SEQ ID NO: 1 - protein, 810 aa, Homo sapiens
MLLLFHSKRMPVAEAPQVAGGQGDGGDGEEAEPEGMFKACEDSKRKARGYLRLVPLFVLLALLVLASAGVLLWYFLGYKAEVMVSQVYSGSLRVLNRHFSQDLTRRESSAFRSETAKAQKMLKELITSTRLGTYYNSSSVYSFGEGPLTCFFWFILQIPEHRRLMLSPEVVQALLVEELLSTVNSSAAVPYRAEYEVDPEGLVILEASVKDIAALNSTLGCYRYSYVGQGQVLRLKGPDHLASSCLWHLQGPKDLMLKLRLEWTLAECRDRLAMYDVAGPLEKRLITSVYGCSRQEPVVEVLASGAIMAVVWKKGLHSYYDPFVLSVQPVVFQACEVNLTLDNRLDSQGVLSTPYFPSYYSPQTHCSWHLTVPSLDYGLALWFDAYALRRQKYDLPCTQGQWTIQNRRLCGLRILQPYAERIPVVATAGITINFTSQISLTGPGVRVHYGLYNQSDPCPGEFLCSVNGLCVPACDGVKDCPNGLDERNCVCRATFQCKEDTCISLPKVCDGQPDCLNGSDEEQCQEGVPCGTFTFQCEDRSCVKKPNPQCDGRPDCRDGSDEEHCDCGLQGPSSRIVGGAVSSEGEWPWQASLQVRGRHICGGALIADRWVITAAHCFQEDSMASTVLWTVFLGKVWQNSRWPGEVSFKVSRLLLHPYHEEDSHDYDVALLQLDHPVVRSAAVRPVCLPARSHFFEPGLHCWITGWGALREGGPISNALQKVDVQLIPQDLCSEVYRYQVTPRMLCAGYRKGKKDACQGDSGGPLVCKALSGRWFLAGLVSWGLGCGRPNYFGVYTRITGVISWIQQVVT

SEQ ID NO: 2 - protein, 228 aa, Homo sapiens
MASTASEIIAFMVSISGWVLVSSTLPTDYWKVSTIDGTVITTATYWANLWKACVTDSTGVSNCKDFPSMLALDGYIQACRGLMIAAVSLGFFGSIFALFGMKCTKVGGSDKAKAKIACLAGIVFILSGLCSMTGCSLYANKITTEFFDPLFVEQKYELGAALFIGWAGASLCIIGGVIFCFSISDNNKTPRYTYNGATSVMSSRTKYHGGEDFKTTNPSKQFDKNAYV